European Patent Application EP 4 501 946 A1, published February 5, 2025. Title: Self-amplifying biologics for targeted therapy. Applicant: LoopLab Bio GmbH. The sequence listing filed with the application follows.

SEQUENCE LISTING (12 sequences)

SEQ ID NO: 1 - DNA, 1995 bp, synthetic construct
  source 1..1995: mol_type = other DNA
atgcacaagggaatccccaaaagctccaaaacccaaacacatacccaacaagaccgccccccacaacccagcaccgaactcgaagagaccaggacctcccgagcacgacacagcacaacatcagctcagcgatccacgcactacgatcctcgaacatcggacagacccgtctcctacaccatgaacaggaccaggtcccgcaagcaaaccagccacagattgaagaacatcccagttcacggaaaccacgaggccaccatccagcacataccagagagtgtctcaaaaggagcgagatcccagatcgaaaggcggcaacccaatgcaatcaactcaggctctcagtgcacctggttagtcctgtggtgcctcggaatggccagtctctttctttgttccaaggctcagatacattggaataatttgtcaactattgggattatcgggactgatagtgtccattacaagatcatgactaggcccagtcaccagtacttggtcataaaactgatgcctaatgtttcacttatagagaattgtaccaaagcagaattaggtgagtatgagaaattattgaattcagtcctcgaaccaatcaaccaagctttgactctaatgaccaagaatgtgaagcccctgcagtcattagggtcaggtaggagacaaaggcgttttgcaggagtggtacttgcaggtgtagctttaggagtggctacagctgcacaaatcactgcaggaatagctttacatcaatccaacctcaatgctcaagcaatccaatctcttagaaccagccttgaacagtctaacaaagctatagaagaaattagggaggctacccaagaaaccgtcattgccgttcagggagtccaggactacgtcaacaacgaactcgtccctgccatgcaacatatgtcatgtgaattagttgggcagagattagggttaagactgcttcggtattatactgagttgttgtcaatatttggcccgagtttacgtgaccctatttcagccgagatatcaattcaggcactgatttatgctcttggaggagaaattcataagatacttgagaagttgggatattctggaagtgatatgattgcaatcttggagagtcgggggataaaaacaaaaataactcatgttgatcttcccgggaaattcatcatcctaagtatctcatacccaactttatcagaagtcaagggggttatagtccacagactggaagcagtttcttacaacataggatcacaagagtggtacaccactgtcccgaggtatattgcaactaatggttacttaatatctaattttgatgagtcatcttgtgtattcgtctcagagtcagccatttgtagccagaactccctgtatcccatgagcccactcttacaacaatgtattaggggcgacacttcatcttgtgctcggaccttggtatctgggactatgggcaacaaatttattctgtcaaaaggtaatatcgtcgcaaattgtgcttctatactatgtaagtgttatagcacaagcacaattattaatcagagtcctgataagttgctgacattcattgcctccgatacctgcccactggttgaaatagatggtgctactatccaagttggaggcaggcaataccctgatatggtatacgaaggcaaagttgccttaggccctgctatatcacttgataggttagatgtaggtacaaacttagggaacgcccttaagaaactggatgatgctaaggtactgatagactcctctaaccagatccttgagacggttaggcgctcttcctttaattttggcagtatagtctacatcctgattgcagtgtgtcttggagggttgatagggatccccgctttaatatgttgctgcagggggcgttgtaacaaaaagggagaacaagttggtatgtcaagaccaggcctaaagcctgatcttacgggaacatcaaaatcctatgtaaggtcgctctaa

SEQ ID NO: 2 - DNA, 1815 bp, synthetic construct
  source 1..1815: mol_type = other DNA
atgtcaccacaacgagaccggataaatgccttctacaaagataacccccatcccaagggaagtaggatagtcattaacagagaacatcttatgattgatagaccttatgttttgctggctgttctgtttgtcatgtttctgagcttgatcgggttgctagccattgcaggcattcgatttcaccaagtatcaactagtaatatggaatttagcagattgctgaaagaggatatggagaaatcagaggccgtacatcaccaagtcatagatgtcttgacaccgctcttcaagattattggagatgagattgggttacggttgccacaaaagctaaacgagatcaaacaatttatccttcaaaagacaaatttcttcaatccgaacagagaattcgacttccgcgatctccactggtgcattaacccgcctagtacggtcaaggtgaattttactaattactgtgagtcaattgggatcagaaaagctattgcatcggcagcaaatcctatccttttatcagccctatctgggggcagaggtgacatattcccaccacacagatgcagtggagctactacttcagtaggcaaagttttccccctatcagtctcattatccatgtctttgatctcaagaacctcagaggtaatcaatatgctgaccgctatctcagacggcgtgtatggcaaaacttacttgctagtgcctgatgatatagaaagagagttcgacactcgagagattcgagtctttgaaatagggttcatcaaaaggtggctgaatgacatgccattactccaaacaaccaactatatggtactcccgaagaattccaaagccaaggtatgtactatagcagtgggtgagttgacactggcttccttgtgtgtagaagagagcactgtattattatatcatgacagcagtggttcacaagatggtattctagtagtgacactggggatattttgggcaacacctatggatcacattgaggaagtgatacctgtcgctcacccatcaatgaagaaaatacatataacaaaccaccgtggttttataaaagattcaattgcaacctggatggtgcctgccctggcctctgagaaacaagaagaacaaaaaggttgtctggagtcagcttgtcaaagaaaaacctaccccatgtgcaaccaagcgtcatgggaacccttcggaggaagacagttgccatcttatgggcggttgacattacctctagatgcaagtgttgaccttcaacttaacatatcgttcacatacggtccggttatactgaatggagatggtatggattattatgaaagcccacttttgaactccggatggcttaccattccccccaaagacggaacaatctctggattgataaacaaagcaggtagaggagaccagttcactgtactcccccatgtgttaacatttgcgcccagggaatcaagtggaaattgttatttacctattcaaacatctcaaattagagatagagatgtcctcattgagtccaatatagtggtgttgcctacacagagtattagatatgtcatagcaacgtatgacatatcacgaagtgatcatgctattgtttattatgtttatgacccaatccggacgatttcttatacgcacccatttagactaactaccaagggtagacctgatttcctaaggattgaatgttttgtgtgggatgacaatttgtggtgtcaccaattttacagattcgaggctgacatcgccaactctacaaccagtgttgagaatttagtccgtataagattctcatgtaaccgttaa

SEQ ID NO: 3 - DNA, 1578 bp, synthetic construct
  source 1..1578: mol_type = other DNA
atggccacacttttaaggagcttagcattgttcaaaagaaacaaggacaaaccacccattacatcaggatccggtggagccatcagaggaatcaaacacattattatagtaccaatccctggagattcctcaattaccactcgatccagacttctggaccggttggtgaggttaattggaaacccggatgtgagcgggcccaaactaacaggggcactaataggtatattatccttatttgtggagtctccaggtcaattgattcagaggatcaccgatgaccctgacgttagcataaggctgttagaggttgtccagagtgaccagtcacaatctggccttaccttcgcatcaagaggtaccaacatggaggatgaggcggaccaatacttttcacatgatgatccaattagtagtgatcaatccaggttcggatggttcgggaacaaggaaatctcagatattgaagtgcaagaccctgagggattcaacatgattctgggtaccatcctagcccaaatttgggtcttgctcgcaaaggcggttacggccccagacacggcagctgattcggagctaagaaggtggataaagtacacccaacaaagaagggtagttggtgaatttagattggagagaaaatggttggatgtggtgaggaacaggattgccgaggacctctccttacgccgattcatggtcgctctaatcctggatatcaagagaacacccggaaacaaacccaggattgctgaaatgatatgtgacattgatacatatatcgtagaggcaggattagccagttttatcctgactattaagtttgggatagaaactatgtatcctgctcttggactgcatgaatttgctggtgagttatccacacttgagtccttgatgaacctttaccagcaaatgggggaaactgcaccctacatggtaatcctggagaactcaattcagaacaagttcagtgcaggatcataccctctgctctggagctatgccatgggagtaggagtggaacttgaaaactccatgggaggtttgaactttggccgatcttactttgatccagcatattttagattagggcaagagatggtaaggaggtcagctggaaaggtcagttccacattggcatctgaactcggtatcactgccgaggatgcaaggcttgtttcagagattgcaatgcatactactgaggacaagatcagtagagcggttggacccagacaagcccaagtatcatttctacacggtgatcaaagtgagaatgagctaccgagattggggggcaaggaagataggagggtcaaacagagtcgaggagaagccagggagagctacagagaaaccgggcccagcagagcaagtgatgcgagagctgcccatcttccaaccggcacacccctagacattgacactgcaacggagtccagccaagatccgcaggacagtcgaaggtcagctgacgccctgcttaggctgcaagccatggcaggaatctcggaagaacaaggctcagacacggacacccctatagtgtacaatgacagaaatcttctagactag

SEQ ID NO: 4 - DNA, 1524 bp, synthetic construct
  source 1..1524: mol_type = other DNA
atggcagaagagcaggcacgccatgtcaaaaacggactggaatgcatccgggctctcaaggccgagcccatcggctcactggccatcgaggaagctatggcagcatggtcagaaatatcagacaacccaggacaggagcgagccacctgcagggaagagaaggcaggcagttcgggtctcagcaaaccatgcctctcagcaattggatcaactgaaggcggtgcacctcgcatccgcggtcagggacctggagagagcgatgacgacgctgaaactttgggaatccccccaagaaatctccaggcatcaagcactgggttacagtgttattacgtttatgatcacagcggtgaagcggttaagggaatccaagatgctgactctatcatggttcaatcaggccttgatggtgatagcaccctctcaggaggagacaatgaatctgaaaacagcgatgtggatattggcgaacctgataccgagggatatgctatcactgaccggggatctgctcccatctctatggggttcagggcttctgatgttgaaactgcagaaggaggggagatccacgagctcctgagactccaatccagaggcaacaactttccgaagcttgggaaaactctcaatgttcctccgcccccggaccccggtagggccagcacttccgggacacccattaaaaagggcacagacgcgagattagcctcatttggaacggagatcgcgtctttattgacaggtggtgcaacccaatgtgctcgaaagtcaccctcggaaccatcagggccaggtgcacctgcggggaatgtccccgagtgtgtgagcaatgccgcactgatacaggagtggacacccgaatctggtaccacaatctccccgagatcccagaataatgaagaagggggagactattatgatgatgagctgttctctgatgtccaagatattaaaacagccttggccaaaatacacgaggataatcagaagataatctccaagctagaatcactgctgttattgaagggagaagttgagtcaattaagaagcagatcaacaggcaaaatatcagcatatccaccctggaaggacacctctcaagcatcatgatcgccattcctggacttgggaaggatcccaacgaccccactgcagatgtcgaaatcaatcccgacttgaaacccatcataggcagagattcaggccgagcactggccgaagttctcaagaaacccgttgccagccgacaactccaaggaatgacaaatggacggaccagttccagaggacagctgctgaaggaatttcagctaaagccgatcgggaaaaagatgagctcagccgtcgggtttgttcctgacaccggccctgcatcacgcagtgtaatccgctccattataaaatccagccggctagaggaggatcggaagcgttacctgatgactctccttgatgatatcaaaggagccaatgatcttgccaagttccaccagatgctgatgaagataataatgaagtag

SEQ ID NO: 5 - DNA, 1008 bp, synthetic construct
  source 1..1008: mol_type = other DNA
atgacagagacctacgacttcgacaagtcggcatgggacatcaaagggtcgatcgctccgatacaacccaccacctacagtgatggcaggctggtgccccaggtcagagtcatagatcctggtctaggcgacaggaaggatgaatgctttatgtacatgtttctgctgggggttgttgaggacagcgattccctagggcctccaatcgggcgagcatttgggttcctgcccttaggtgttggcagatccacagcaaagcccgaaaaactcctcaaagaggccactgagcttgacatagttgttagacgtacagcagggctcaatgaaaaactggtgttctacaacaacaccccactaactctcctcacaccttggagaaaggtcctaacaacagggagtgtcttcaacgcaaaccaagtgtgcaatgcggttaatctgataccgctcgataccccgcagaggttccgtgttgtttatatgagcatcacccgtctttcggataacgggtattacaccgttcctagaagaatgctggaattcagatcggtcaatgcagtggccttcaacctgctggtgacccttaggattgacaaggcgataggccctgggaagatcatcgacaatacagagcaacttcctgaggcaacatttatggtccacatcgggaacttcaggagaaagaagagtgaagtctactctgccgattattgcaaaatgaaaatcgaaaagatgggcctggtttttgcacttggtgggatagggggcaccagtcttcacattagaagcacaggcaaaatgagcaagactctccatgcacaactcgggttcaagaagaccttatgttacccgctgatggatatcaatgaagaccttaatcgattactctggaggagcagatgcaagatagtaagaatccaggcagttttgcagccatcagttcctcaagaattccgcatttacgacgacgtgatcataaatgatgaccaaggactattcaaagttctgtag

SEQ ID NO: 6 - DNA, 6552 bp, synthetic construct
  source 1..6552: mol_type = other DNA
atggactcgctatctgtcaaccagatcttataccctgaagttcacctagatagcccgatagttaccaataagatagtagccatcctggagtatgctcgagtccctcacgcttacagcctggaggaccctacactgtgtcagaacatcaagcaccgcctaaaaaacggattttccaaccaaatgattataaacaatgtggaagttgggaatgtcatcaagtccaagcttaggagttatccggcccactctcatattccatatccaaattgtaatcaggatttatttaacatagaagacaaagagtcaacgaggaagatccgtgaactcctcaaaaaggggaattcgctgtactccaaagtcagtgataaggttttccaatgcttaagggacactaactcacggcttggcctaggctccgaattgagggaggacatcaaggagaaagttattaacttgggagtttacatgcacagctcccagtggtttgagccctttctgttttggtttacagtcaagactgagatgaggtcagtgattaaatcacaaacccatacttgccataggaggagacacacacctgtattcttcactggtagttcagttgagttgctaatctctcgtgaccttgttgctataatcagtaaagagtctcaacatgtatattacctgacatttgaactggttttgatgtattgtgatgtcatagaggggaggttaatgacagagaccgctatgactattgatgctaggtatacagagcttctaggaagagtcagatacatgtggaaactgatagatggtttcttccctgcactcgggaatccaacttatcaaattgtagccatgctggagcctctttcacttgcttacctgcagctgagggatataacagtagaactcagaggtgctttccttaaccactgctttactgaaatacatgatgttcttgaccaaaacgggttttctgatgaaggtacttatcatgagttaactgaagctctagattacattttcataactgatgacatacatctgacaggggagattttctcatttttcagaagtttcggccaccccagacttgaagcagtaacggctgctgaaaatgttaggaaatacatgaatcagcctaaagtcattgtgtatgagactctgatgaaaggtcatgccatattttgtggaatcataatcaacggctatcgtgacaggcacggaggcagttggccaccgctgaccctccccctgcatgctgcagacacaatccggaatgctcaagcttcaggtgaagggttaacacatgagcagtgcgttgataactggaaatcttttgctggagtgaaatttggctgctttatgcctcttagcctggatagtgatctgacaatgtacctaaaggacaaggcacttgctgctctccaaagggaatgggattcagtttacccgaaagagttcctgcgttacgaccctcccaagggaaccgggtcacggaggcttgtagatgttttccttaatgattcgagctttgacccatatgatgtgataatgtatgttgtaagtggagcttacctccatgaccctgagttcaacctgtcttacagcctgaaagaaaaggagatcaaggaaacaggtagactttttgctaaaatgacttacaaaatgagggcatgccaagtgattgctgaaaatctaatctcaaacgggattggcaaatattttaaggacaatgggatggccaaggatgagcacgatttgactaaggcactccacactctagctgtctcaggagtccccaaagatctcaaagaaagtcacaggggggggccagtcttaaaaacctactcccgaagcccagtccacacaagtaccaggaacgtgagagcagcaaaagggtttatagggttccctcaagtaattcggcaggaccaagacactgatcatccggagaatatggaagcttacgagacagtcagtgcatttatcacgactgatctcaagaagtactgccttaattggagatatgagaccatcagcttgtttgcacagaggctaaatgagatttacggattgccctcatttttccagtggctgcataagaggcttgagacctctgtcctgtatgtaagtgaccctcattgcccccccgaccttgacgcccatatcccgttatataaagtccccaatgatcaaatcttcattaagtaccctatgggaggtatagaagggtattgtcagaagctgtggaccatcagcaccattccctatctatacctggctgcttatgagagcggagtaaggattgcttcgttagtgcaaggggacaatcagaccatagccgtaacaaaaagggtacccagcacatggccctacaaccttaagaaacgggaagctgctagagtaactagagattactttgtaattcttaggcaaaggctacatgatattggccatcacctcaaggcaaatgagacaattgtttcatcacatttttttgtctattcaaaaggaatatattatgatgggctacttgtgtcccaatcactcaagagcatcgcaagatgtgtattctggtcagagactatagttgatgaaacaagggcagcatgcagtaatattgctacaacaatggctaaaagcatcgagagaggttatgaccgttaccttgcatattccctgaacgtcctaaaagtgatacagcaaattctgatctctcttggcttcacaatcaattcaaccatgacccgggatgtagtcatacccctcctcacaaacaacgacctcttaataaggatggcactgttgcccgctcctattggggggatgaattatctgaatatgagcaggctgtttgtcagaaacatcggtgatccagtaacatcatcaattgctgatctcaagagaatgattctcgcctcactaatgcctgaagagaccctccatcaagtaatgacacaacaaccgggggactcttcattcctagactgggctagcgacccttactcagcaaatcttgtatgtgtccagagcatcactagactcctcaagaacataactgcaaggtttgtcctgatccatagtccaaacccaatgttaaaaggattattccatgatgacagtaaagaagaggacgagggactggcggcattcctcatggacaggcatattatagtacctagggcagctcatgaaatcctggatcatagtgtcacaggggcaagagagtctattgcaggcatgctggataccacaaaaggcttgattcgagccagcatgaggaagggggggttaacctctcgagtgataaccagattgtccaattatgactatgaacaattcagagcagggatggtgctattgacaggaagaaagagaaatgtcctcattgacaaagagtcatgttcagtgcagctggcgagagctctaagaagccatatgtgggcgaggctagctcgaggacggcctatttacggccttgaggtccctgatgtactagaatctatgcgaggccaccttattcggcgtcatgagacatgtgtcatctgcgagtgtggatcagtcaactacggatggttttttgtcccctcgggttgccaactggatgatattgacaaggaaacatcatccttgagagtcccatatattggttctaccactgatgagagaacagacatgaagcttgccttcgtaagagccccaagtcgatccttgcgatctgctgttagaatagcaacagtgtactcatgggcttacggtgatgatgatagctcttggaacgaagcctggttgttggctaggcaaagggccaatgtgagcctggaggagctaagggtgatcactcccatctcaacttcgactaatttagcgcataggttgagggatcgtagcactcaagtgaaatactcaggtacatcccttgtccgagtggcgaggtataccacaatctccaacgacaatctctcatttgtcatatcagataagaaggttgatactaactttatataccaacaaggaatgcttctagggttgggtgttttagaaacattgtttcgactcgagaaagataccggatcatctaacacggtattacatcttcacgtcgaaacagattgttgcgtgatcccgatgatagatcatcccaggatacccagctcccgcaagctagagctgagggcagagctatgtaccaacccattgatatatgataatgcacctttaattgacagagatgcaacaaggctatacacccagagccataggaggcaccttgtggaatttgttacatggtccacaccccaactatatcacattttagctaagtccacagcactatctatgattgacctggtaacaaaatttgagaaggaccatatgaatgaaatttcagctctcataggggatgacgatatcaatagtttcataactgagtttctgctcatagagccaagattattcactatctacttgggccagtgtgcggccatcaattgggcatttgatgtacattatcatagaccatcagggaaatatcagatgggtgagctgttgtcatcgttcctttctagaatgagcaaaggagtgtttaaggtgcttgtcaatgctctaagccacccaaagatctacaagaaattctggcattgtggtattatagagcctatccatggtccttcacttgatgctcaaaacttgcacacaactgtgtgcaacatggtttacacatgctatatgacctacctcgacctgttgttgaatgaagagttagaagagttcacatttctcttgtgtgaaagcgacgaggatgtagtaccggacagattcgacaacatccaggcaaaacacttatgtgttctggcagatttgtactgtcaaccagggacctgcccaccaattcgaggtctaagaccggtagagaaatgtgcagttctaaccgaccatatcaaggcagaggctatgttatctccagcaggatcttcgtggaacataaatccaattattgtagaccattactcatgctctctgacttatctccggcgaggatcgatcaaacagataagattgagagttgatccaggattcattttcgacgccctcgctgaggtaaatgtcagtcagccaaagatcggcagcaacaacatctcaaatatgagcatcaaggctttcagacccccacacgatgatgttgcaaaattgctcaaagatatcaacacaagcaagcacaatcttcccatttcagggggcaatctcgccaattatgaaatccatgctttccgcagaatcgggttgaactcatctgcttgctacaaagctgttgagatatcaacattaattaggagatgccttgagccaggggaggacggcttgttcttgggtgagggatcgggttctatgttgatcacttataaagagatacttaaactaaacaagtgcttctataatagtggggtttccgccaattctagatctggtcaaagggaattagcaccctatccctccgaagttggccttgtcgaacacagaatgggagtaggtaatattgtcaaagtgctctttaacgggaggcccgaagtcacgtgggtaggcagtgtagattgcttcaatttcatagttagtaatatccctacctctagtgtggggtttatccattcagatatagagaccttgcctgacaaagatactatagagaagctagaggaattggcagccatcttatcgatggctctgctcctgggcaaaataggatcaatactggtgattaagcttatgcctttcagcggggattttgttcagggatttataagttatgtagggtctcattatagagaagtgaaccttgtataccctagatacagcaacttcatctctactgaatcttatttggttatgacagatctcaaggctaaccggctaatgaatcctgaaaagattaagcagcagataattgaatcatctgtgaggacttcacctggacttataggtcacatcctatccattaagcaactaagctgcatacaagcaattgtgggagacgcagttagtagaggtgatatcaatcctactctgaaaaaacttacacctatagagcaggtgctgatcaattgcgggttggcaattaacggacctaagctgtgcaaagaattgatccaccatgatgttgcctcagggcaagatggattgcttaattctatactcatcctctacagggagttggcaagattcaaagacaaccaaagaagtcaacaagggatgttccacgcttaccccgtattggtaagtagcaggcaacgagaacttatatctaggatcacccgcaaattctgggggcacattcttctttactccgggaacaaaaagttgataaataagtttatccagaatctcaagtccggctatctgatactagacttacaccagaatatcttcgttaagaatctatccaagtcagagaaacagattattatgacggggggtttgaaacgtgagtgggtttttaaggtaacagtcaaggagaccaaagaatggtataagttagtcggatacagtgccctgattaaggactaa

SEQ ID NO: 7 - DNA, 304 bp, Cytomegalovirus
  source 1..304: mol_type = other DNA
cctggcattatgcccagtacatgaccttatgggactttcctacttggcagtacatctacgtattagtcatcgctattaccatggtgatgcggttttggcagtacatcaatgggcgtggatagcggtttgactcacggggatttccaagtctccaccccattgacgtcaatgggagtttgttttggcaccaaaatcaacgggactttccaaaatgtcgtaacaactccgccccattgacgcaaatgggcggtaggcgtgtacggtgggaggtctatataagcagagctcgtttagtgaaccgtgg

SEQ ID NO: 8 - DNA, 11 bp, synthetic construct
  source 1..11: mol_type = other DNA
caggtccacac

SEQ ID NO: 9 - DNA, 11 bp, synthetic construct
  source 1..11: mol_type = other DNA
attaagaaaaa

SEQ ID NO: 10 - DNA, 52 bp, Measles morbillivirus
  source 1..52: mol_type = other DNA
accaaacaaagttgggtaaggatagttcaatcaatgatcatcttctagtgca

SEQ ID NO: 11 - DNA, 37 bp, Measles morbillivirus
  source 1..37: mol_type = other DNA
tgaaaatacgaagtttctattcccagctttgtctggt

SEQ ID NO: 12 - DNA, 1572 bp, synthetic construct
  source 1..1572: mol_type = other DNA
atgaagtgccttttgtacttagcctttttattcattggggtgaattgcaagttcaccatagtttttccacacaaccaaaaaggaaactggaaaaatgttccttctaattaccattattgcccgtcaagctcagatttaaattggcataatgacttaataggcacagccttacaagtcaaaatgcccaagagtcacaaggctattcaagcagacggttggatgtgtcatgcttccaaatgggtcactacttgtgatttccgctggtatggaccgaagtatataacacattccatccgatccttcactccatctgtagaacaatgcaaggaaagcattgaacaaacgaaacaaggaacttggctgaatccaggcttccctcctcaaagttgtggatatgcaactgtgacggatgccgaagcagtgattgtccaggtgactcctcaccatgtgctggttgatgaatacacaggagaatgggttgattcacagttcatcaacggaaaatgcagcaattacatatgccccactgtccataactctacaacctggcattctgactataaggtcaaagggctatgtgattctaacctcatttccatggacatcaccttcttctcagaggacggagagctatcatccctgggaaaggagggcacagggttcagaagtaactactttgcttatgaaactggaggcaaggcctgcaaaatgcaatactgcaagcattggggagtcagactcccatcaggtgtctggttcgagatggctgataaggatctctttgctgcagccagattccctgaatgcccagaagggtcaagtatctctgctccatctcagacctcagtggatgtaagtctaattcaggacgttgagaggatcttggattattccctctgccaagaaacctggagcaaaatcagagcgggtcttccaatctctccagtggatctcagctatcttgctcctaaaaacccaggaaccggtcctgctttcaccataatcaatggtaccctaaaatactttgagaccagatacatcagagtcgatattgctgctccaatcctctcaagaatggtcggaatgatcagtggaactaccacagaaagggaactgtgggatgactgggcaccatatgaagacgtggaaattggacccaatggagttctgaggaccagttcaggatataagtttcctttatacatgattggacatggtatgttggactccgatcttcatcttagctcaaaggctcaggtgttcgaacatcctcacattcaagacgctgcttcgcaacttcctgatgatgagagtttattttttggtgatactgggctatccaaaaatccaatcgagcttgtagaaggttggttcagtagttggaaaagctctattgcctcttttttctttatcatagggttaatcattggactattcttggttctccgagttggtatccatctttgctgcagggggcgttgtaacaaaaagggagaacaagttggtatgtcaagaccaggcctaaagcctgatcttacgggaacatcaaaatcctatgtaaggtcgctctaa